European Patent Specification EP 3 853 384 B1, published November 26, 2025. Title: UTILISATION DE SONDES POUR LA DETECTION D ALGUES TOXIQUES, PROCEDE DE DETECTION ET KITS CORRESPONDANTS. Applicant: MICROBIA ENVIRONNEMENT. The sequence listing filed with the application follows.

SEQUENCE LISTING (129 sequences)

SEQ ID NO: 1 - DNA, 32 bp, Artificial sequence
  Sonde
  DNA (1)..(32): b = c, g ou t
aaacactctgatttcctcaaagtaaabgttct

SEQ ID NO: 2 - DNA, 30 bp, Artificial sequence
  Sonde
ctaatgtattcaaggccaaacacctgcttg

SEQ ID NO: 3 - DNA, 24 bp, Artificial sequence
  Sonde
cacgatcttgattattattccatg

SEQ ID NO: 4 - DNA, 29 bp, Artificial sequence
  Sonde
gaggagtgtgactcgtcaaatatataccg

SEQ ID NO: 5 - DNA, 25 bp, Artificial sequence
  Sonde
accacccactttgcattccaatgcc

SEQ ID NO: 6 - DNA, 19 bp, Artificial sequence
  Sonde
ttctgcaaccaacgaccac

SEQ ID NO: 7 - DNA, 20 bp, Artificial sequence
  Sonde
aacctttcccccaagatagg

SEQ ID NO: 8 - DNA, 24 bp, Artificial sequence
  Sonde
gttgaacacatcagtgtagcgcgc

SEQ ID NO: 9 - DNA, 25 bp, Artificial sequence
  Sonde
cctttccaggcaaggttgcaaactc

SEQ ID NO: 10 - DNA, 25 bp, Artificial sequence
  Sonde
gatgcattttttcaagattacccaa

SEQ ID NO: 11 - DNA, 36 bp, Artificial sequence
  Sonde
aatcaagtctgtttactttgtgtttagcaaatacaa

SEQ ID NO: 12 - DNA, 25 bp, Artificial sequence
  Sonde
gcaagcactacaatctcactgagga

SEQ ID NO: 13 - DNA, 26 bp, Artificial sequence
  Sonde
cacttgcagccaaaacccattgttaa

SEQ ID NO: 14 - DNA, 30 bp, Artificial sequence
  Sonde
ccattcatatgcaagggtaataatttgcag

SEQ ID NO: 15 - DNA, 25 bp, Artificial sequence
  Sonde
cattccaatgcccacaggcaaatta

SEQ ID NO: 16 - DNA, 27 bp, Artificial sequence
  Sonde
caaatcacaaatcattgcaaacacatg

SEQ ID NO: 17 - DNA, 27 bp, Artificial sequence
  Sonde
cctgggttggttctgtaactaatgacc

SEQ ID NO: 18 - DNA, 25 bp, Artificial sequence
  Sonde
gaatcaccaaggttccaagcagagc

SEQ ID NO: 19 - DNA, 28 bp, Artificial sequence
  Sonde
gttgccatgtaattcattcagtcattat

SEQ ID NO: 20 - DNA, 34 bp, Artificial sequence
  Sonde
atcaagtctgtttactttgtgttcagcaaataca

SEQ ID NO: 21 - DNA, 25 bp, Artificial sequence
  Sonde
caagtgcaacactcccaccaagcaa

SEQ ID NO: 22 - DNA, 26 bp, Artificial sequence
  Sonde
acccacagcccaaagctcttgtcaag

SEQ ID NO: 23 - DNA, 25 bp, Artificial sequence
  Sonde
caagtctgtttactttgtgttcagc

SEQ ID NO: 24 - DNA, 25 bp, Artificial sequence
  Sonde
agtgcaacactcccaccaagcaaat

SEQ ID NO: 25 - DNA, 26 bp, Artificial sequence
  Sonde
ccacagcccaaagctcttgtcaagca

SEQ ID NO: 26 - DNA, 28 bp, Artificial sequence
  Sonde
aaacactctgatttcctcaaagtaaatg

SEQ ID NO: 27 - DNA, 25 bp, Artificial sequence
  Sonde
gtattcaaggccaaacacctgcttg

SEQ ID NO: 28 - DNA, 29 bp, Artificial sequence
  Sonde
cacgatcttgattattattccatgctaat

SEQ ID NO: 29 - DNA, 25 bp, Artificial sequence
  Sonde
atgctcatcgcaaccacagcaaagc

SEQ ID NO: 30 - DNA, 28 bp, Artificial sequence
  Sonde
ttgaggatggacagccctgcagccagac

SEQ ID NO: 31 - DNA, 24 bp, Artificial sequence
  Sonde
tcgtcaagatctgtgcagaaggtt

SEQ ID NO: 32 - DNA, 25 bp, Artificial sequence
  Sonde
cacttgcgttgtggcagcaaccaat

SEQ ID NO: 33 - DNA, 25 bp, Artificial sequence
  Sonde
ccttgcagcatgtgacaatctcacc

SEQ ID NO: 34 - DNA, 26 bp, Artificial sequence
  Sonde
cctgcagccagacaaacactaaagct

SEQ ID NO: 35 - DNA, 30 bp, Artificial sequence
  Sonde
tacgcacaagcataacaacacacattcaca

SEQ ID NO: 36 - DNA, 27 bp, Artificial sequence
  Sonde
acatcgccagttggtaccatgcaattc

SEQ ID NO: 37 - DNA, 33 bp, Artificial sequence
  Sonde
attcgtttattatgaatcaccacgagaccaagc

SEQ ID NO: 38 - DNA, 23 bp, Artificial sequence
  Sonde
  DNA (1)..(23): r = a ou g y = c ou t k = g ou t m = a ou c
rattcacamatygccakcacact

SEQ ID NO: 39 - DNA, 21 bp, Artificial sequence
  Sonde
tgcgttgtggcagcaaccaat

SEQ ID NO: 40 - DNA, 25 bp, Artificial sequence
  Sonde
cagactttccacggcaacaattagg

SEQ ID NO: 41 - DNA, 30 bp, Artificial sequence
  Sonde
aactaaacattgctgcagtccgaattattc

SEQ ID NO: 42 - DNA, 25 bp, Artificial sequence
  Sonde
ccttcctctaagtgataaggttcac

SEQ ID NO: 43 - DNA, 23 bp, Artificial sequence
  Sonde
caccagactttccacggcaacgc

SEQ ID NO: 44 - DNA, 26 bp, Artificial sequence
  Sonde
tcaggaactgaacactgctgcagtcc

SEQ ID NO: 45 - DNA, 27 bp, Artificial sequence
  Sonde
cttctccttcctctaagtgttaaggtt

SEQ ID NO: 46 - DNA, 24 bp, Artificial sequence
  Sonde
ccacggcaacgttcaggaactaaa

SEQ ID NO: 47 - DNA, 27 bp, Artificial sequence
  Sonde
cattgctgcagtccgaattattcaccg

SEQ ID NO: 48 - DNA, 27 bp, Artificial sequence
  Sonde
tctaagtgataaggttcaccagacttt

SEQ ID NO: 49 - DNA, 29 bp, Artificial sequence
  Sonde
  DNA (1)..(29): y = c ou t
tgcacgacaacytaatgccacacagattc

SEQ ID NO: 50 - DNA, 26 bp, Artificial sequence
  Sonde
  DNA (1)..(26): r = a ou g
cacccaaacatggcagaccagtacar

SEQ ID NO: 51 - DNA, 36 bp, Artificial sequence
  Sonde
gaatttcacctctgacaatggaatacaaataccccc

SEQ ID NO: 52 - DNA, 33 bp, Artificial sequence
  Sonde
aactgtccctcttaatcattaccttagtgcgca

SEQ ID NO: 53 - DNA, 30 bp, Artificial sequence
  Sonde
ggacacaccacaaatccaactacgagcttt

SEQ ID NO: 54 - DNA, 40 bp, Artificial sequence
  Sonde
ttaactgcaacaactttaatatacgctattggagctggaa

SEQ ID NO: 55 - DNA, 26 bp, Artificial sequence
  Sonde
aatcactcaaagagcaaaggccgact

SEQ ID NO: 56 - DNA, 23 bp, Artificial sequence
  Sonde
gacaacgactcactctaccaggc

SEQ ID NO: 57 - DNA, 23 bp, Artificial sequence
  Sonde
ggacgggagtctcaccctctcag

SEQ ID NO: 58 - DNA, 25 bp, Artificial sequence
  Sonde
gcaatcccaaacaactcgactcgtt

SEQ ID NO: 59 - DNA, 25 bp, Artificial sequence
  Sonde
aacccaaactcacgaaagctcacag

SEQ ID NO: 60 - DNA, 25 bp, Artificial sequence
  Sonde
ctgcgctcttccaaagggatcaacc

SEQ ID NO: 61 - DNA, 25 bp, Artificial sequence
  Sonde
cgcccaagccacaagtggccgggga

SEQ ID NO: 62 - DNA, 24 bp, Artificial sequence
  Sonde
gcaatcagaacccatcctagtcct

SEQ ID NO: 63 - DNA, 31 bp, Artificial sequence
  Sonde
gcgcggaagatgttaccaagcaacgtcagct

SEQ ID NO: 64 - DNA, 25 bp, Artificial sequence
  Sonde
catggcaagaaacacaacacacatt

SEQ ID NO: 65 - DNA, 24 bp, Artificial sequence
  Sonde
agctctagcatttccacgggtatc

SEQ ID NO: 66 - DNA, 29 bp, Artificial sequence
  Sonde
catgtaagagtgaaccaccaaataaattg

SEQ ID NO: 67 - DNA, 25 bp, Artificial sequence
  Sonde
taagttgggtaggagcgcatgtatt

SEQ ID NO: 68 - DNA, 24 bp, Artificial sequence
  Sonde
acaccccaattgcctcgtaggcag

SEQ ID NO: 69 - DNA, 29 bp, Artificial sequence
  Sonde
ggagctgcaaccaaccaccaatttttcag

SEQ ID NO: 70 - DNA, 22 bp, Artificial sequence
  Sonde
tcctcgtctgcgtgtcagggct

SEQ ID NO: 71 - DNA, 24 bp, Artificial sequence
  Sonde
ccgcaaatgagttctgccaaggct

SEQ ID NO: 72 - DNA, 24 bp, Artificial sequence
  Sonde
attcactcacccgtagacgagcta

SEQ ID NO: 73 - DNA, 24 bp, Artificial sequence
  Sonde
gcaaccagacacgaaagaaacagt

SEQ ID NO: 74 - DNA, 25 bp, Artificial sequence
  Sonde
ggacgaggaaccctcatccagattt

SEQ ID NO: 75 - DNA, 27 bp, Artificial sequence
  Sonde
acaacatgagctcttcccgcttcactc

SEQ ID NO: 76 - DNA, 25 bp, Artificial sequence
  Sonde
gcacgcatctctagactacaattcg

SEQ ID NO: 77 - DNA, 30 bp, Artificial sequence
  Sonde
atgttccgcaaaaagcatccagcatacaaa

SEQ ID NO: 78 - DNA, 25 bp, Artificial sequence
  Sonde
cagtccaagccacgacagagaatgt

SEQ ID NO: 79 - DNA, 25 bp, Artificial sequence
  Sonde
cacaggcaacggcaagatggaacct

SEQ ID NO: 80 - DNA, 25 bp, Artificial sequence
  Sonde
ctttcacaaacagacttagccctgg

SEQ ID NO: 81 - DNA, 25 bp, Artificial sequence
  Sonde
gggttatcaccgtccatgacactgt

SEQ ID NO: 82 - DNA, 25 bp, Artificial sequence
  Sonde
cgctacaacatccaaggcaagaacc

SEQ ID NO: 83 - DNA, 24 bp, Artificial sequence
  Sonde
caccgccccgctttcgctggaata

SEQ ID NO: 84 - DNA, 25 bp, Artificial sequence
  Sonde
gaaggtgatcattgctgcgtgcgac

SEQ ID NO: 85 - DNA, 28 bp, Artificial sequence
  Sonde
gaaacatcacaccgaacaaatcacagcc

SEQ ID NO: 86 - DNA, 30 bp, Artificial sequence
  Sonde
gcatttttaaaagattacccaatcctgtcg

SEQ ID NO: 87 - DNA, 26 bp, Artificial sequence
  Sonde
gacaaggtcgtaaactcgttgagtgc

SEQ ID NO: 88 - DNA, 26 bp, Artificial sequence
  Sonde
ttgcaataatctatccccatcacgat

SEQ ID NO: 89 - DNA, 27 bp, Artificial sequence
  Sonde
cgtatagttaacggcctccaatctcta

SEQ ID NO: 90 - DNA, 27 bp, Artificial sequence
  Sonde
gtcggcatggtttatggttaagactag

SEQ ID NO: 91 - DNA, 26 bp, Artificial sequence
  Sonde
gatttctcataaggtgctgaaggagt

SEQ ID NO: 92 - DNA, 22 bp, Artificial sequence
  Sonde
acatctacgcccctgctggcag

SEQ ID NO: 93 - DNA, 26 bp, Artificial sequence
  Sonde
cgcgtcgagagattacaattcgtggc

SEQ ID NO: 94 - DNA, 26 bp, Artificial sequence
  Sonde
cagtgattcgcttttccaagcggctt

SEQ ID NO: 95 - DNA, 25 bp, Artificial sequence
  Sonde
caacgttcaggatctgaacactgcg

SEQ ID NO: 96 - DNA, 24 bp, Artificial sequence
  Sonde
gcagtccgaattattcaccggatc

SEQ ID NO: 97 - DNA, 24 bp, Artificial sequence
  Sonde
taaggttcactaaactttccactg

SEQ ID NO: 98 - DNA, 25 bp, Artificial sequence
  Sonde
gcagtgcgaccagacacacagtgag

SEQ ID NO: 99 - DNA, 28 bp, Artificial sequence
  Sonde
cagttcaaaaatgagttcaactggggac

SEQ ID NO: 100 - DNA, 27 bp, Artificial sequence
  Sonde
gcagaagattgcaagcaagcacacgga

SEQ ID NO: 101 - DNA, 25 bp, Artificial sequence
  Sonde
cttcatgcagagcagaagatcgcag

SEQ ID NO: 102 - DNA, 27 bp, Artificial sequence
  Sonde
gcaagcacatgaagcagtgctaccaga

SEQ ID NO: 103 - DNA, 30 bp, Artificial sequence
  Sonde
tgtcaaggacatgctcctggcaccaacaac

SEQ ID NO: 104 - DNA, 25 bp, Artificial sequence
  Sonde
cgttcaggatctgaacactgcggca

SEQ ID NO: 105 - DNA, 25 bp, Artificial sequence
  Sonde
gtccgaattattcaccggatcactc

SEQ ID NO: 106 - DNA, 24 bp, Artificial sequence
  Sonde
ggttcactaaactttccactgcaa

SEQ ID NO: 107 - DNA, 26 bp, Artificial sequence
  Sonde
cggagcagtgcgaccagacacacagt

SEQ ID NO: 108 - DNA, 29 bp, Artificial sequence
  Sonde
gagcagttcaaaaatgagttcaatgggga

SEQ ID NO: 109 - DNA, 31 bp, Artificial sequence
  Sonde
catgccaagcagaagattgcaagcaagcaca

SEQ ID NO: 110 - DNA, 24 bp, Artificial sequence
  Sonde
agcagaagatcgcaggcaagcaca

SEQ ID NO: 111 - DNA, 29 bp, Artificial sequence
  Sonde
tgaagcagtgctaccagacacacagagag

SEQ ID NO: 112 - DNA, 30 bp, Artificial sequence
  Sonde
atgctcctggcaccaacaaccttcatgcag

SEQ ID NO: 113 - DNA, 25 bp, Artificial sequence
  Sonde
agcagaagattgcaagcaagcacac

SEQ ID NO: 114 - DNA, 35 bp, Artificial sequence
  Sonde
ggagcagtgcgaccagacacacagtgagcagttca

SEQ ID NO: 115 - DNA, 31 bp, Artificial sequence
  Sonde
catgctcctggcactagcaaccttcatgcca

SEQ ID NO: 116 - DNA, 25 bp, Artificial sequence
  Sonde
acatgctcctggcactagcaacctt

SEQ ID NO: 117 - DNA, 27 bp, Artificial sequence
  Sonde
catgccaagcagaagattgcaagcaag

SEQ ID NO: 118 - DNA, 25 bp, Artificial sequence
  Sonde
tttcgtcatcgttcttatgtcaagg

SEQ ID NO: 119 - DNA, 25 bp, Artificial sequence
  Sonde
ggcaaacaggactgtcaccctcatt

SEQ ID NO: 120 - DNA, 29 bp, Artificial sequence
  Sonde
agtgctcttttccaagaggcttacatctg

SEQ ID NO: 121 - DNA, 22 bp, Artificial sequence
  Sonde
ccgtgcatggaagacgacagat

SEQ ID NO: 122 - DNA, 25 bp, Artificial sequence
  Sonde
ggactgtcaccctcattagtgctct

SEQ ID NO: 123 - DNA, 26 bp, Artificial sequence
  Sonde
tttccaagaggcttacatctgcaccc

SEQ ID NO: 124 - DNA, 25 bp, Artificial sequence
  Sonde
catggaagacgacagatggcaaaca

SEQ ID NO: 125 - DNA, 25 bp, Artificial sequence
  Sonde
ctgcacccccattggcaacgcatct

SEQ ID NO: 126 - DNA, 25 bp, Artificial sequence
  Sonde
ccagactacaactcaaggctaccag

SEQ ID NO: 127 - DNA, 25 bp, Artificial sequence
  Sonde
gtgctattttccaagaggcttacat

SEQ ID NO: 128 - DNA, 27 bp, Artificial sequence
  Sonde
acgacaagaacagtgcgtttccccgaa

SEQ ID NO: 129 - DNA, 25 bp, Artificial sequence
  Sonde
ggaccacgactgagcacgcaccttt